European Patent Specification EP 4 153 310 B1, published February 18, 2026. Title: COMPOUNDS FOR THE TREATMENT OF ENDOTHELIITIS IN CONTEXT OF VIRALLY CAUSED DISEASES. Applicant: Johann Wolfang Goethe-Universitt Frankfurt am Main Julius-Maximilians-Universitt Würzburg. The sequence listing filed with the application follows.

SEQUENCE LISTING (28 sequences)

SEQ ID NO: 1 - protein, 28 aa, Artificial Sequence
  fibrin-derived peptide B Beta 15-42
GHRPLDKKREEAPSLRPAPPPISGGGYR

SEQ ID NO: 2 - protein, 29 aa, Artificial Sequence
  fibrin-derived peptide B Beta 15-42 derivative
  misc_feature (5)..(5): any amino acid residue
  misc_feature (6)..(6): any amino acid residue
  misc_feature (7)..(7): any amino acid residue
  misc_feature (8)..(8): any amino acid residue
  misc_feature (9)..(9): any amino acid residue
  misc_feature (10)..(10): any amino acid residue
  misc_feature (11)..(11): any amino acid residue
  misc_feature (12)..(12): any amino acid residue
  misc_feature (14)..(14): any amino acid residue
  misc_feature (15)..(15): any amino acid residue
  misc_feature (16)..(16): any amino acid residue
  misc_feature (18)..(18): any amino acid residue
  misc_feature (22)..(22): any amino acid residue
  misc_feature (23)..(23): any amino acid residue
  misc_feature (24)..(24): any amino acid residue
  misc_feature (25)..(25): any amino acid residue
  misc_feature (29)..(29): OR1, wherein R1 is H or a C1-C10 alkyl group, or NR2R3, wherein R2 and R3 are hydrogen, a C1-C10 alkyl group, or -PEG5-60K, or a residue NH-Y1-Z-PEG5-60K, wherein Y1 is a chemical bond or S, C, K and R, and Z is a spacer
GHRPXXXXXXXXPXXXPXPPPXXXXGYRX

SEQ ID NO: 3 - protein, 29 aa, Artificial Sequence
  fibrin-derived peptide B Beta 15-42 derivative
  misc_feature (5)..(5): any amino acid residue
  misc_feature (6)..(6): any amino acid residue
  misc_feature (7)..(7): any amino acid residue
  misc_feature (8)..(8): any amino acid residue
  misc_feature (9)..(9): any amino acid residue
  misc_feature (10)..(10): any amino acid residue
  misc_feature (11)..(11): any amino acid residue
  misc_feature (12)..(12): any amino acid residue
  misc_feature (14)..(14): any amino acid residue
  misc_feature (15)..(15): any amino acid residue
  misc_feature (16)..(16): any amino acid residue
  misc_feature (18)..(18): any amino acid residue
  misc_feature (22)..(22): any amino acid residue
  misc_feature (23)..(23): any amino acid residue
  misc_feature (24)..(24): any amino acid residue
  DISULFID (25)..(25): cysteine residue forms a disulfide bond with a second peptide having the same sequence
  MISC_FEATURE (29)..(29): OR1, NR2R3, -PEG5-60K-CO-, NH-Y1-Z-PEG5-60K or NH-CH(CONH2)-(CH2)4-NH-CO-Y2-PEG5-60K, R1, R2, R3, R4 or R5 is H or a C1-C10 alkyl group, or R2 and R3 is -PEG5-60K, Y1 is a single bond or S, C, K and R, and Z is a spacer, Y2 is O or NH
GHRPXXXXXXXXPXXXPXPPPXXXCGYRX

SEQ ID NO: 4 - protein, 29 aa, Artificial Sequence
  fibrin-derived peptide B Beta 15-42 derivative
  misc_feature (5)..(5): any amino acid residue
  misc_feature (6)..(6): any amino acid residue
  misc_feature (7)..(7): any amino acid residue
  misc_feature (8)..(8): any amino acid residue
  misc_feature (9)..(9): any amino acid residue
  misc_feature (10)..(10): any amino acid residue
  misc_feature (11)..(11): any amino acid residue
  misc_feature (12)..(12): any amino acid residue
  misc_feature (14)..(14): any amino acid residue
  misc_feature (15)..(15): any amino acid residue
  misc_feature (16)..(16): any amino acid residue
  misc_feature (18)..(18): Xaa can be any naturally occurring amino acid
  misc_feature (22)..(22): any amino acid residue
  misc_feature (23)..(23): any amino acid residue
  DISULFID (24)..(24)
  misc_feature (25)..(25): any amino acid residue
  misc_feature (29)..(29): OR1, NR2R3, -PEG5-60K-CO-, NH-Y1-Z-PEG5-60K or NH-CH(CONH2)-(CH2)4-NH-CO-Y2-PEG5-60K, R1, R2, R3, R4 or R5 is H or a C1-C10 alkyl group, or R2 and R3 is -PEG5-60K, Y1 is a single bond or S, C, K and R, and Z is a spacer, Y2 is O or NH
GHRPXXXXXXXXPXXXPXPPPXXCXGYRX

SEQ ID NO: 5 - protein, 30 aa, Artificial Sequence
  fibrin-derived peptide B Beta 15-42 derivative
  misc_feature (5)..(5): any amino acid residue
  misc_feature (6)..(6): any amino acid residue
  misc_feature (7)..(7): any amino acid residue
  misc_feature (8)..(8): Xaa can be any naturally occurring amino acid
  misc_feature (9)..(9): any amino acid residue
  misc_feature (10)..(10): any amino acid residue
  misc_feature (11)..(11): any amino acid residue
  misc_feature (12)..(12): any amino acid residue
  misc_feature (14)..(14): any amino acid residue
  misc_feature (15)..(15): any amino acid residue
  misc_feature (16)..(16): any amino acid residue
  misc_feature (18)..(18): any amino acid residue
  misc_feature (22)..(22): any amino acid residue
  misc_feature (23)..(23): any amino acid residue
  misc_feature (24)..(24): any amino acid residue
  misc_feature (25)..(25): any amino acid residue
  BINDING (29)..(29): dimer via lysine residue bound to -CO-(CH2)m-Y3-(CH2)m-CO-, Y3 is -N-CO-(CH2)n-NH-CO-Z-PEG5-60K or -N-CO-(CH2)n-NH-CO-CH(NH-CO-Z-PEG5-60K)-(CH2)4-NH-CO-Z-PEG5-60K, m is 1, 2, 3 or 4, Z is NH or O
  misc_feature (30)..(30): is OH or NH2
GHRPXXXXXXXXPXXXPXPPPXXXXGYRKX

SEQ ID NO: 6 - protein, 23 aa, Artificial Sequence
  fibrin-derived peptide B Beta 15-42 derivative
  misc_feature (5)..(5): any amino acid residue
  misc_feature (6)..(6): any amino acid residue
  misc_feature (8)..(8): any amino acid residue
  misc_feature (9)..(9): any amino acid residue
  misc_feature (10)..(10): any amino acid residue
  misc_feature (12)..(12): any amino acid residue
  misc_feature (16)..(16): any amino acid residue
  misc_feature (17)..(17): any amino acid residue
  misc_feature (18)..(18): any amino acid residue
  misc_feature (19)..(19): any amino acid residue
  misc_feature (20)..(20): is a chemical bond or G
  misc_feature (21)..(21): is a chemical bond or Y
  misc_feature (22)..(22): is a chemical bond or R
  misc_feature (23)..(23): OR1, wherein R1 is H or a C1-C10 alkyl group, or NR2R3, wherein R2 and R3 are hydrogen, a C1-C10 alkyl group, or -PEG5-60K, or a residue NH-Y1-Z-PEG5-60K, wherein Y1 is a chemical bond or S, C, K and R, and Z is a spacer
GHRPXXPXXXPXPPPXXXXXXXX

SEQ ID NO: 7 - protein, 29 aa, Artificial Sequence
  fibrin-derived peptide B Beta 15-42 derivative
  misc_feature (5)..(5): any amino acid residue
  misc_feature (6)..(6): any amino acid residue
  misc_feature (7)..(7): any amino acid residue
  misc_feature (8)..(8): any amino acid residue
  misc_feature (9)..(9): any amino acid residue
  misc_feature (10)..(10): any amino acid residue
  misc_feature (11)..(11): any amino acid residue
  misc_feature (12)..(12): any amino acid residue
  misc_feature (14)..(14): any amino acid residue
  misc_feature (15)..(15): any amino acid residue
  misc_feature (16)..(16): any amino acid residue
  misc_feature (18)..(18): any amino acid residue
  misc_feature (22)..(22): any amino acid residue
  misc_feature (23)..(23): any amino acid residue
  misc_feature (24)..(24): any amino acid residue
  misc_feature (25)..(25): any amino acid residue
  misc_feature (26)..(26): is a chemical bond or G
  misc_feature (27)..(27): is a chemical bond or Y
  misc_feature (28)..(28): is a chemical bond or R
  misc_feature (29)..(29): OR1, wherein R1 is H or a C1-C10 alkyl group, or NR2R3, wherein R2 and R3 are hydrogen, a C1-C10 alkyl group, or -PEG5-60K, or a residue NH-Y1-Z-PEG5-60K, wherein Y1 is a chemical bond or S, C, K and R, and Z is a spacer
GHRPXXXXXXXXPXXXPXPPPXXXXXXXX

SEQ ID NO: 8 - protein, 16 aa, Artificial Sequence
  fibrin-derived peptide B Beta 15-42 derivative
  misc_feature (5)..(5): any amino acid residue
  misc_feature (6)..(6): any amino acid residue
  misc_feature (7)..(7): any amino acid residue
  misc_feature (8)..(8): an amino acid residue or a peptidomimetic element
  misc_feature (9)..(9): any amino acid residue
  misc_feature (10)..(10): any amino acid residue
  misc_feature (11)..(11): any amino acid residue
  misc_feature (12)..(12): any amino acid residue
  misc_feature (13)..(13): any amino acid residue or a bond
  misc_feature (14)..(14): any amino acid residue or a bond
  misc_feature (15)..(15): any amino acid residue or a bond
  misc_feature (16)..(16): OR1, wherein R1 is H or a C1-C10 alkyl group, or NR2R3, wherein R2 and R3 are hydrogen, a C1-C10 alkyl group, or -PEG5-60K, or a residue NH-Y1-Z-PEG5-60K, wherein Y1 is a chemical bond or S, C, K and R, and Z is a spacer
GHRPXXXXXXXXXXXX

SEQ ID NO: 9 - protein, 28 aa, Artificial Sequence
  fibrin-derived peptide B Beta 15-42 derivative
  misc_feature (28)..(28): modified to have a Cterminal amino group
GHRPLDKKREEAPSLRPAPPPISGGGYR

SEQ ID NO: 10 - protein, 29 aa, Artificial Sequence
  fibrin-derived peptide B Beta 15-42 derivative
  misc_feature (29)..(29): comprising a C-terminal -(S-CH2-CO-NH-PEG20K)-OH
GHRPLDKKREEAPSLRPAPPPISGGGYRC

SEQ ID NO: 11 - protein, 29 aa, Artificial Sequence
  fibrin-derived peptide B Beta 15-42 derivative
  misc_feature (29)..(29): comprising a C-terminal -(S-CH2-CO-NH-PEG20K)-amid
GHRPLDKKREEAPSLRPAPPPISGGGYRC

SEQ ID NO: 12 - protein, 29 aa, Artificial Sequence
  fibrin-derived peptide B Beta 15-42 derivative
  misc_feature (26)..(26): X is -(S-CH2-CO-NH-PEG20K)-
  misc_feature (29)..(29): comprising a C-terminal amide group
GHRPLDKKREEAPSLRPAPPPISGCXGYR

SEQ ID NO: 13 - protein, 28 aa, Artificial Sequence
  fibrin-derived peptide B Beta 15-42 derivative
  DISULFID (25)..(25): homodimeric peptide having a disulfide bond at position 25
GHRPLDKKREEAPSLRPAPPPISGCGYR

SEQ ID NO: 14 - protein, 28 aa, Artificial Sequence
  fibrin-derived peptide B Beta 15-42 derivative
  DISULFID (24)..(24): homodimeric peptide having a disulfide bond at position 24
GHRPLDKKREEAPSLRPAPPPISCGGYR

SEQ ID NO: 15 - protein, 29 aa, Artificial Sequence
  fibrin-derived peptide B Beta 15-42 derivative
  misc_feature (25)..(25): homodimer bound at position 25 via (S-CH2)2CH-CH2-CO-NH-PEG5-30K to each other
  misc_feature (29)..(29): OR1, wherein R1 is H or a C1-C10 alkyl group, or NR2R3, wherein R2 and R3 are hydrogen, a C1-C10 alkyl group, or -PEG5-60K, or a residue NH-Y1-Z-PEG5-60K, wherein Y1 is a chemical bond or S, C, K and R, and Z is a spacer
GHRPLDKKREEAPSLRPAPPPISGCGYRX

SEQ ID NO: 16 - protein, 29 aa, Artificial Sequence
  fibrin-derived peptide B Beta 15-42 derivative
  misc_feature (24)..(24): homodimer bound at position 25 via (S-CH2)2CH-CH2-CO-NH-PEG5-30K to each other
  misc_feature (29)..(29): OR1, wherein R1 is H or a C1-C10 alkyl group, or NR2R3, wherein R2 and R3 are hydrogen, a C1-C10 alkyl group, or -PEG5-60K, or a residue NH-Y1-Z-PEG5-60K, wherein Y1 is a chemical bond or S, C, K and R, and Z is a spacer
GHRPLDKKREEAPSLRPAPPPISCGGYRX

SEQ ID NO: 17 - protein, 22 aa, Artificial Sequence
  fibrin-derived peptide B Beta 15-42 derivative
  misc_feature (22)..(22): comprising a terminal OH group
GHRPLAPSLRPAPPPISGGGYR

SEQ ID NO: 18 - protein, 22 aa, Artificial Sequence
  fibrin-derived peptide B Beta 15-42 derivative
  misc_feature (22)..(22): comprising a C-terminal NH2 group
GHRPLAPSLRPAPPPISGGGYR

SEQ ID NO: 19 - protein, 23 aa, Artificial Sequence
  fibrin-derived peptide B Beta 15-42 derivative
  misc_feature (23)..(23): comprising a C-terminal -(S-succinimide-PEG20K)-OH
GHRPLAPSLRPAPPPISGGGYRC

SEQ ID NO: 20 - protein, 23 aa, Artificial Sequence
  fibrin-derived peptide B Beta 15-42 derivative
  misc_feature (23)..(23): comprising a C-terminal -(S-succinimido-PEG20K)-amide
GHRPLAPSLRPAPPPISGGGYRC

SEQ ID NO: 21 - protein, 25 aa, Artificial Sequence
  fibrin-derived peptide B Beta 15-42 derivative
  misc_feature (25)..(25): comprising a C-terminal -OH
GHRPLDKKREEAPSLRPAPPPISGG

SEQ ID NO: 22 - protein, 25 aa, Artificial Sequence
  fibrin-derived peptide B Beta 15-42 derivative
  misc_feature (25)..(25): comprising a C-terminal -NH2
GHRPLDKKREEAPSLRPAPPPISGG

SEQ ID NO: 23 - protein, 26 aa, Artificial Sequence
  fibrin-derived peptide B Beta 15-42 derivative
  misc_feature (26)..(26): comprising a C-terminal -OH
GHRPLDKKREEAPSLRPAPPPISGGG

SEQ ID NO: 24 - protein, 26 aa, Artificial Sequence
  fibrin-derived peptide B Beta 15-42 derivative
  misc_feature (26)..(26): comprising a C-terminal -NH2
GHRPLDKKREEAPSLRPAPPPISGGG

SEQ ID NO: 25 - protein, 15 aa, Artificial Sequence
  fibrin-derived peptide B Beta 15-42 derivative
  misc_feature (8)..(8): X is -(1S,2R)Achc-
GHRPLDKXISGGGYR

SEQ ID NO: 26 - protein, 15 aa, Artificial Sequence
  fibrin-derived peptide B Beta 15-42 derivative
  misc_feature (8)..(8): X is Acdn
GHRPLDKXISGGGYR

SEQ ID NO: 27 - protein, 15 aa, Artificial Sequence
  fibrin-derived peptide B Beta 15-42 derivative
  misc_feature (8)..(8): X is -(cis-4-Acha)-
GHRPLDKXISGGGYR

SEQ ID NO: 28 - protein, 15 aa, Artificial Sequence
  fibrin-derived peptide B Beta 15-42 derivative
  misc_feature (8)..(8): X is -Haic-
GHRPLDKXISGGGYR